European Patent Application EP 4 119 945 A1, published January 18, 2023. Title: HIGHLY SENSITIVE IMMUNOCONJUGATE, PREPARING METHOD THEREOF, IN VITRO DIAGNOSTIC REAGENT AND IN VITRO DIAGNOSTIC KIT INCLUDING THE SAME. Applicant: BioMetrix Technology INC. The sequence listing filed with the application follows.

SEQUENCE LISTING (4 sequences)

SEQ ID NO: 1 - DNA, 26 bp, Artificial Sequence
  Sequence of DNA fragment included in immunoconjugate for in vitro diagnosis
tttatatttataccttgcgagcgcgg

SEQ ID NO: 2 - DNA, 26 bp, Artificial Sequence
  Sequence of DNA fragment included in immunoconjugate for in vitro diagnosis
tttatattttggccacactgtccatt

SEQ ID NO: 3 - DNA, 26 bp, Artificial Sequence
  Sequence of DNA fragment included in immunoconjugate for in vitro diagnosis
tttatatttccgcgctcgcaaggtat

SEQ ID NO: 4 - DNA, 26 bp, Artificial Sequence
  Sequence of DNA fragment included in immunoconjugate for in vitro diagnosis
tttatatttaatggacagtgtggcca